European Patent Application EP 4 768 582 A2, published July 1, 2026. Title: 一种靶向AGT基因表达的siRNA及其缀合物和用途. Applicant: 成都先衍生物技术有限公司. The sequence listing filed with the application follows.

SEQUENCE LISTING (351 sequences)

SEQ ID NO: 1 - RNA, 21 nt, synthetic construct
  source 1..21: mol_type = other RNA
gaggtgctgaacagcattttt

SEQ ID NO: 2 - RNA, 20 nt, synthetic construct
  source 1..20: mol_type = other RNA
gctcccaccttttcttctaa

SEQ ID NO: 3 - RNA, 19 nt, synthetic construct
  source 1..19: mol_type = other RNA
caccttttcttctaatgaa

SEQ ID NO: 4 - RNA, 20 nt, synthetic construct
  source 1..20: mol_type = other RNA
ccagcttttcttctaatgaa

SEQ ID NO: 5 - RNA, 20 nt, synthetic construct
  source 1..20: mol_type = other RNA
cgagcttttcttctaatgaa

SEQ ID NO: 6 - RNA, 20 nt, synthetic construct
  source 1..20: mol_type = other RNA
agagtctatccaacagctta

SEQ ID NO: 7 - RNA, 20 nt, synthetic construct
  source 1..20: mol_type = other RNA
agagtctactcaacagctta

SEQ ID NO: 8 - RNA, 20 nt, synthetic construct
  source 1..20: mol_type = other RNA
agagtctacctaacagctta

SEQ ID NO: 9 - RNA, 20 nt, synthetic construct
  source 1..20: mol_type = other RNA
gggtctcattttccagcaat

SEQ ID NO: 10 - RNA, 20 nt, synthetic construct
  source 1..20: mol_type = other RNA
gggtctcacttttcagcaat

SEQ ID NO: 11 - RNA, 20 nt, synthetic construct
  source 1..20: mol_type = other RNA
gggtctcactttctagcaat

SEQ ID NO: 12 - RNA, 20 nt, synthetic construct
  source 1..20: mol_type = other RNA
aggtgctaaacagcattttt

SEQ ID NO: 13 - RNA, 20 nt, synthetic construct
  source 1..20: mol_type = other RNA
aggtgctgaatagcattttt

SEQ ID NO: 14 - RNA, 20 nt, synthetic construct
  source 1..20: mol_type = other RNA
aggtgctgaacagtattttt

SEQ ID NO: 15 - RNA, 20 nt, synthetic construct
  source 1..20: mol_type = other RNA
aggtgctgaacagcattttt

SEQ ID NO: 16 - RNA, 20 nt, synthetic construct
  source 1..20: mol_type = other RNA
aggtgctgaacagcatttta

SEQ ID NO: 17 - RNA, 19 nt, synthetic construct
  source 1..19: mol_type = other RNA
ggtgctgaacagcattttt

SEQ ID NO: 18 - RNA, 19 nt, synthetic construct
  source 1..19: mol_type = other RNA
ggtgctgaacagcatttta

SEQ ID NO: 19 - RNA, 20 nt, synthetic construct
  source 1..20: mol_type = other RNA
gggtctcactttccagcaat

SEQ ID NO: 20 - RNA, 20 nt, synthetic construct
  source 1..20: mol_type = other RNA
agagtctacccaacagctta

SEQ ID NO: 21 - RNA, 20 nt, synthetic construct
  source 1..20: mol_type = other RNA
tctcccaccttttcttctaa

SEQ ID NO: 22 - RNA, 20 nt, synthetic construct
  source 1..20: mol_type = other RNA
ctcccaccttttcttctaaa

SEQ ID NO: 23 - RNA, 20 nt, synthetic construct
  source 1..20: mol_type = other RNA
ccaccttttcttctaatgaa

SEQ ID NO: 24 - RNA, 21 nt, synthetic construct
  source 1..21: mol_type = other RNA
agggtctcactttccagcaat

SEQ ID NO: 25 - RNA, 19 nt, synthetic construct
  source 1..19: mol_type = other RNA
ggtctcactttccagcaat

SEQ ID NO: 26 - RNA, 21 nt, synthetic construct
  source 1..21: mol_type = other RNA
cagagtctacccaacagctta

SEQ ID NO: 27 - RNA, 19 nt, synthetic construct
  source 1..19: mol_type = other RNA
gagtctacccaacagctta

SEQ ID NO: 28 - RNA, 19 nt, synthetic construct
  source 1..19: mol_type = other RNA
ctcccaccttttcttctaa

SEQ ID NO: 29 - RNA, 20 nt, synthetic construct
  source 1..20: mol_type = other RNA
ccaccttttcttctaatgat

SEQ ID NO: 30 - RNA, 20 nt, synthetic construct
  source 1..20: mol_type = other RNA
ctcccactttttcttctaaa

SEQ ID NO: 31 - RNA, 20 nt, synthetic construct
  source 1..20: mol_type = other RNA
ctaccttttcttctaatgaa

SEQ ID NO: 32 - RNA, 21 nt, synthetic construct
  source 1..21: mol_type = other RNA
gaggtgctgaacagcatttta

SEQ ID NO: 33 - RNA, 21 nt, synthetic construct
  source 1..21: mol_type = other RNA
gcggatgagagagagcccaca

SEQ ID NO: 34 - RNA, 21 nt, synthetic construct
  source 1..21: mol_type = other RNA
cggatgagagagagcccacag

SEQ ID NO: 35 - RNA, 21 nt, synthetic construct
  source 1..21: mol_type = other RNA
gagagagagcccacagagtct

SEQ ID NO: 36 - RNA, 21 nt, synthetic construct
  source 1..21: mol_type = other RNA
agcccacagagtctacccaat

SEQ ID NO: 37 - RNA, 21 nt, synthetic construct
  source 1..21: mol_type = other RNA
cggatgagagagagcccacaa

SEQ ID NO: 38 - RNA, 21 nt, synthetic construct
  source 1..21: mol_type = other RNA
gcccacagagtctacccaaca

SEQ ID NO: 39 - RNA, 19 nt, synthetic construct
  source 1..19: mol_type = other RNA
ccacagagtctacccaaca

SEQ ID NO: 40 - RNA, 21 nt, synthetic construct
  source 1..21: mol_type = other RNA
cccacagagtctacccaacaa

SEQ ID NO: 41 - RNA, 19 nt, synthetic construct
  source 1..19: mol_type = other RNA
cacagagtctacccaacaa

SEQ ID NO: 42 - RNA, 19 nt, synthetic construct
  source 1..19: mol_type = other RNA
tcccaccttttcttctaaa

SEQ ID NO: 43 - RNA, 20 nt, synthetic construct
  source 1..20: mol_type = other RNA
cacccccagtctcccacctt

SEQ ID NO: 44 - RNA, 20 nt, synthetic construct
  source 1..20: mol_type = other RNA
acccccagtctcccaccttt

SEQ ID NO: 45 - RNA, 20 nt, synthetic construct
  source 1..20: mol_type = other RNA
cccccagtctcccacctttt

SEQ ID NO: 46 - RNA, 20 nt, synthetic construct
  source 1..20: mol_type = other RNA
ccccagtctcccaccttttt

SEQ ID NO: 47 - RNA, 20 nt, synthetic construct
  source 1..20: mol_type = other RNA
cccagtctcccaccttttct

SEQ ID NO: 48 - RNA, 20 nt, synthetic construct
  source 1..20: mol_type = other RNA
ccagtctcccaccttttctt

SEQ ID NO: 49 - RNA, 20 nt, synthetic construct
  source 1..20: mol_type = other RNA
cagtctcccaccttttcttt

SEQ ID NO: 50 - RNA, 20 nt, synthetic construct
  source 1..20: mol_type = other RNA
agtctcccaccttttcttct

SEQ ID NO: 51 - RNA, 20 nt, synthetic construct
  source 1..20: mol_type = other RNA
gtctcccaccttttcttcta

SEQ ID NO: 52 - RNA, 20 nt, synthetic construct
  source 1..20: mol_type = other RNA
tcccaccttttcttctaata

SEQ ID NO: 53 - RNA, 20 nt, synthetic construct
  source 1..20: mol_type = other RNA
cccaccttttcttctaatga

SEQ ID NO: 54 - RNA, 20 nt, synthetic construct
  source 1..20: mol_type = other RNA
caccttttcttctaatgagt

SEQ ID NO: 55 - RNA, 20 nt, synthetic construct
  source 1..20: mol_type = other RNA
accttttcttctaatgagtt

SEQ ID NO: 56 - RNA, 20 nt, synthetic construct
  source 1..20: mol_type = other RNA
ccttttcttctaatgagtca

SEQ ID NO: 57 - RNA, 20 nt, synthetic construct
  source 1..20: mol_type = other RNA
cttttcttctaatgagtcga

SEQ ID NO: 58 - RNA, 20 nt, synthetic construct
  source 1..20: mol_type = other RNA
ttttcttctaatgagtcgat

SEQ ID NO: 59 - RNA, 20 nt, synthetic construct
  source 1..20: mol_type = other RNA
tttcttctaatgagtcgact

SEQ ID NO: 60 - RNA, 19 nt, synthetic construct
  source 1..19: mol_type = other RNA
acccccagtctcccacctt

SEQ ID NO: 61 - RNA, 19 nt, synthetic construct
  source 1..19: mol_type = other RNA
cccccagtctcccaccttt

SEQ ID NO: 62 - RNA, 19 nt, synthetic construct
  source 1..19: mol_type = other RNA
ccccagtctcccacctttt

SEQ ID NO: 63 - RNA, 19 nt, synthetic construct
  source 1..19: mol_type = other RNA
cccagtctcccaccttttt

SEQ ID NO: 64 - RNA, 19 nt, synthetic construct
  source 1..19: mol_type = other RNA
ccagtctcccaccttttct

SEQ ID NO: 65 - RNA, 19 nt, synthetic construct
  source 1..19: mol_type = other RNA
cagtctcccaccttttctt

SEQ ID NO: 66 - RNA, 19 nt, synthetic construct
  source 1..19: mol_type = other RNA
agtctcccaccttttcttt

SEQ ID NO: 67 - RNA, 19 nt, synthetic construct
  source 1..19: mol_type = other RNA
gtctcccaccttttcttct

SEQ ID NO: 68 - RNA, 19 nt, synthetic construct
  source 1..19: mol_type = other RNA
tctcccaccttttcttcta

SEQ ID NO: 69 - RNA, 19 nt, synthetic construct
  source 1..19: mol_type = other RNA
cccaccttttcttctaata

SEQ ID NO: 70 - RNA, 19 nt, synthetic construct
  source 1..19: mol_type = other RNA
ccaccttttcttctaatga

SEQ ID NO: 71 - RNA, 19 nt, synthetic construct
  source 1..19: mol_type = other RNA
accttttcttctaatgagt

SEQ ID NO: 72 - RNA, 19 nt, synthetic construct
  source 1..19: mol_type = other RNA
ccttttcttctaatgagtt

SEQ ID NO: 73 - RNA, 19 nt, synthetic construct
  source 1..19: mol_type = other RNA
cttttcttctaatgagtca

SEQ ID NO: 74 - RNA, 19 nt, synthetic construct
  source 1..19: mol_type = other RNA
ttttcttctaatgagtcga

SEQ ID NO: 75 - RNA, 19 nt, synthetic construct
  source 1..19: mol_type = other RNA
tttcttctaatgagtcgat

SEQ ID NO: 76 - RNA, 19 nt, synthetic construct
  source 1..19: mol_type = other RNA
ttcttctaatgagtcgact

SEQ ID NO: 77 - RNA, 21 nt, synthetic construct
  source 1..21: mol_type = other RNA
tcacccccagtctcccacctt

SEQ ID NO: 78 - RNA, 21 nt, synthetic construct
  source 1..21: mol_type = other RNA
cacccccagtctcccaccttt

SEQ ID NO: 79 - RNA, 21 nt, synthetic construct
  source 1..21: mol_type = other RNA
acccccagtctcccacctttt

SEQ ID NO: 80 - RNA, 21 nt, synthetic construct
  source 1..21: mol_type = other RNA
cccccagtctcccaccttttt

SEQ ID NO: 81 - RNA, 21 nt, synthetic construct
  source 1..21: mol_type = other RNA
ccccagtctcccaccttttct

SEQ ID NO: 82 - RNA, 21 nt, synthetic construct
  source 1..21: mol_type = other RNA
cccagtctcccaccttttctt

SEQ ID NO: 83 - RNA, 21 nt, synthetic construct
  source 1..21: mol_type = other RNA
ccagtctcccaccttttcttt

SEQ ID NO: 84 - RNA, 21 nt, synthetic construct
  source 1..21: mol_type = other RNA
cagtctcccaccttttcttct

SEQ ID NO: 85 - RNA, 21 nt, synthetic construct
  source 1..21: mol_type = other RNA
agtctcccaccttttcttcta

SEQ ID NO: 86 - RNA, 21 nt, synthetic construct
  source 1..21: mol_type = other RNA
ctcccaccttttcttctaata

SEQ ID NO: 87 - RNA, 21 nt, synthetic construct
  source 1..21: mol_type = other RNA
tcccaccttttcttctaatga

SEQ ID NO: 88 - RNA, 21 nt, synthetic construct
  source 1..21: mol_type = other RNA
ccaccttttcttctaatgagt

SEQ ID NO: 89 - RNA, 21 nt, synthetic construct
  source 1..21: mol_type = other RNA
caccttttcttctaatgagtt

SEQ ID NO: 90 - RNA, 21 nt, synthetic construct
  source 1..21: mol_type = other RNA
accttttcttctaatgagtca

SEQ ID NO: 91 - RNA, 21 nt, synthetic construct
  source 1..21: mol_type = other RNA
ccttttcttctaatgagtcga

SEQ ID NO: 92 - RNA, 21 nt, synthetic construct
  source 1..21: mol_type = other RNA
cttttcttctaatgagtcgat

SEQ ID NO: 93 - RNA, 21 nt, synthetic construct
  source 1..21: mol_type = other RNA
ttttcttctaatgagtcgact

SEQ ID NO: 94 - RNA, 20 nt, synthetic construct
  source 1..20: mol_type = other RNA
gtttctccttggtctaagta

SEQ ID NO: 95 - RNA, 20 nt, synthetic construct
  source 1..20: mol_type = other RNA
cctgtggtcctcccacgctt

SEQ ID NO: 96 - RNA, 20 nt, synthetic construct
  source 1..20: mol_type = other RNA
acatacaccccttccacctt

SEQ ID NO: 97 - RNA, 20 nt, synthetic construct
  source 1..20: mol_type = other RNA
ggtgtacatacaccccttct

SEQ ID NO: 98 - RNA, 20 nt, synthetic construct
  source 1..20: mol_type = other RNA
gtggagggtctcactttcca

SEQ ID NO: 99 - RNA, 20 nt, synthetic construct
  source 1..20: mol_type = other RNA
tacgtccacttccaagggaa

SEQ ID NO: 100 - RNA, 20 nt, synthetic construct
  source 1..20: mol_type = other RNA
cagtctcccaccttttctct

SEQ ID NO: 101 - RNA, 20 nt, synthetic construct
  source 1..20: mol_type = other RNA
tgtggtcctcccacgctctt

SEQ ID NO: 102 - RNA, 23 nt, synthetic construct
  source 1..23: mol_type = other RNA
aaaaatgctgttcagcacctccc

SEQ ID NO: 103 - RNA, 22 nt, synthetic construct
  source 1..22: mol_type = other RNA
ttagaagaaaaggtgggagcct

SEQ ID NO: 104 - RNA, 21 nt, synthetic construct
  source 1..21: mol_type = other RNA
ttcattagaagaaaaggtgtt

SEQ ID NO: 105 - RNA, 22 nt, synthetic construct
  source 1..22: mol_type = other RNA
ttcattagaagaaaaggtggtt

SEQ ID NO: 106 - RNA, 22 nt, synthetic construct
  source 1..22: mol_type = other RNA
taagctgttgggtagactctgt

SEQ ID NO: 107 - RNA, 22 nt, synthetic construct
  source 1..22: mol_type = other RNA
attgctggaaagtgagaccctc

SEQ ID NO: 108 - RNA, 22 nt, synthetic construct
  source 1..22: mol_type = other RNA
aaaaatgctgttcagcacctcc

SEQ ID NO: 109 - RNA, 22 nt, synthetic construct
  source 1..22: mol_type = other RNA
aaaaatgctgttcagcaccttt

SEQ ID NO: 110 - RNA, 22 nt, synthetic construct
  source 1..22: mol_type = other RNA
taaaatgctgttcagcaccttt

SEQ ID NO: 111 - RNA, 21 nt, synthetic construct
  source 1..21: mol_type = other RNA
aaaaatgctgttcagcacctt

SEQ ID NO: 112 - RNA, 21 nt, synthetic construct
  source 1..21: mol_type = other RNA
taaaatgctgttcagcacctt

SEQ ID NO: 113 - RNA, 22 nt, synthetic construct
  source 1..22: mol_type = other RNA
attgctggaaagtgagaccctt

SEQ ID NO: 114 - RNA, 22 nt, synthetic construct
  source 1..22: mol_type = other RNA
taagctgttgggtagactcttt

SEQ ID NO: 115 - RNA, 22 nt, synthetic construct
  source 1..22: mol_type = other RNA
ttagaagaaaaggtgggagatt

SEQ ID NO: 116 - RNA, 22 nt, synthetic construct
  source 1..22: mol_type = other RNA
tttagaagaaaaggtgggagtt

SEQ ID NO: 117 - RNA, 23 nt, synthetic construct
  source 1..23: mol_type = other RNA
attgctggaaagtgagaccctcc

SEQ ID NO: 118 - RNA, 21 nt, synthetic construct
  source 1..21: mol_type = other RNA
attgctggaaagtgagaccct

SEQ ID NO: 119 - RNA, 21 nt, synthetic construct
  source 1..21: mol_type = other RNA
aaaaatgctgttcagcacctc

SEQ ID NO: 120 - RNA, 23 nt, synthetic construct
  source 1..23: mol_type = other RNA
taagctgttgggtagactctgtg

SEQ ID NO: 121 - RNA, 21 nt, synthetic construct
  source 1..21: mol_type = other RNA
taagctgttgggtagactctg

SEQ ID NO: 122 - RNA, 22 nt, synthetic construct
  source 1..22: mol_type = other RNA
taaaatgctgttcagcacctcc

SEQ ID NO: 123 - RNA, 21 nt, synthetic construct
  source 1..21: mol_type = other RNA
taaaatgctgttcagcacctc

SEQ ID NO: 124 - RNA, 22 nt, synthetic construct
  source 1..22: mol_type = other RNA
ttagaagaaaaggtgggagact

SEQ ID NO: 125 - RNA, 22 nt, synthetic construct
  source 1..22: mol_type = other RNA
tttagaagaaaaggtgggagac

SEQ ID NO: 126 - RNA, 21 nt, synthetic construct
  source 1..21: mol_type = other RNA
ttagaagaaaaggtgggagtt

SEQ ID NO: 127 - RNA, 22 nt, synthetic construct
  source 1..22: mol_type = other RNA
ttcattagaagaaaaggtgggg

SEQ ID NO: 128 - RNA, 22 nt, synthetic construct
  source 1..22: mol_type = other RNA
atcattagaagaaaaggtggtt

SEQ ID NO: 129 - RNA, 23 nt, synthetic construct
  source 1..23: mol_type = other RNA
taaaatgctgttcagcacctccc

SEQ ID NO: 130 - RNA, 23 nt, synthetic construct
  source 1..23: mol_type = other RNA
tgtgggctctctctcatccgctt

SEQ ID NO: 131 - RNA, 23 nt, synthetic construct
  source 1..23: mol_type = other RNA
ctgtgggctctctctcatccgct

SEQ ID NO: 132 - RNA, 23 nt, synthetic construct
  source 1..23: mol_type = other RNA
agactctgtgggctctctctcgg

SEQ ID NO: 133 - RNA, 23 nt, synthetic construct
  source 1..23: mol_type = other RNA
attgggtagactctgtgggctct

SEQ ID NO: 134 - RNA, 23 nt, synthetic construct
  source 1..23: mol_type = other RNA
ttgtgggctctctctcatccggg

SEQ ID NO: 135 - RNA, 23 nt, synthetic construct
  source 1..23: mol_type = other RNA
tgttgggtagactctgtgggctc

SEQ ID NO: 136 - RNA, 21 nt, synthetic construct
  source 1..21: mol_type = other RNA
tgttgggtagactctgtgggc

SEQ ID NO: 137 - RNA, 19 nt, synthetic construct
  source 1..19: mol_type = other RNA
tgttgggtagactctgtgg

SEQ ID NO: 138 - RNA, 23 nt, synthetic construct
  source 1..23: mol_type = other RNA
ttgttgggtagactctgtgggct

SEQ ID NO: 139 - RNA, 21 nt, synthetic construct
  source 1..21: mol_type = other RNA
ttgttgggtagactctgtggg

SEQ ID NO: 140 - RNA, 19 nt, synthetic construct
  source 1..19: mol_type = other RNA
ttgttgggtagactctgtg

SEQ ID NO: 141 - RNA, 21 nt, synthetic construct
  source 1..21: mol_type = other RNA
tttagaagaaaaggtgggatt

SEQ ID NO: 142 - RNA, 22 nt, synthetic construct
  source 1..22: mol_type = other RNA
aaggtgggagactgggggtgac

SEQ ID NO: 143 - RNA, 22 nt, synthetic construct
  source 1..22: mol_type = other RNA
aaaggtgggagactgggggtga

SEQ ID NO: 144 - RNA, 22 nt, synthetic construct
  source 1..22: mol_type = other RNA
aaaaggtgggagactgggggtg

SEQ ID NO: 145 - RNA, 22 nt, synthetic construct
  source 1..22: mol_type = other RNA
aaaaaggtgggagactgggggt

SEQ ID NO: 146 - RNA, 22 nt, synthetic construct
  source 1..22: mol_type = other RNA
agaaaaggtgggagactggggg

SEQ ID NO: 147 - RNA, 22 nt, synthetic construct
  source 1..22: mol_type = other RNA
aagaaaaggtgggagactgggg

SEQ ID NO: 148 - RNA, 22 nt, synthetic construct
  source 1..22: mol_type = other RNA
aaagaaaaggtgggagactggg

SEQ ID NO: 149 - RNA, 22 nt, synthetic construct
  source 1..22: mol_type = other RNA
agaagaaaaggtgggagactgg

SEQ ID NO: 150 - RNA, 22 nt, synthetic construct
  source 1..22: mol_type = other RNA
tagaagaaaaggtgggagactg

SEQ ID NO: 151 - RNA, 22 nt, synthetic construct
  source 1..22: mol_type = other RNA
tattagaagaaaaggtgggaga

SEQ ID NO: 152 - RNA, 22 nt, synthetic construct
  source 1..22: mol_type = other RNA
tcattagaagaaaaggtgggag

SEQ ID NO: 153 - RNA, 22 nt, synthetic construct
  source 1..22: mol_type = other RNA
actcattagaagaaaaggtggg

SEQ ID NO: 154 - RNA, 22 nt, synthetic construct
  source 1..22: mol_type = other RNA
aactcattagaagaaaaggtgg

SEQ ID NO: 155 - RNA, 22 nt, synthetic construct
  source 1..22: mol_type = other RNA
tgactcattagaagaaaaggtg

SEQ ID NO: 156 - RNA, 22 nt, synthetic construct
  source 1..22: mol_type = other RNA
tcgactcattagaagaaaaggt

SEQ ID NO: 157 - RNA, 22 nt, synthetic construct
  source 1..22: mol_type = other RNA
atcgactcattagaagaaaagg

SEQ ID NO: 158 - RNA, 22 nt, synthetic construct
  source 1..22: mol_type = other RNA
agtcgactcattagaagaaaag

SEQ ID NO: 159 - RNA, 21 nt, synthetic construct
  source 1..21: mol_type = other RNA
aaggtgggagactgggggtga

SEQ ID NO: 160 - RNA, 21 nt, synthetic construct
  source 1..21: mol_type = other RNA
aaaggtgggagactgggggtg

SEQ ID NO: 161 - RNA, 21 nt, synthetic construct
  source 1..21: mol_type = other RNA
aaaaggtgggagactgggggt

SEQ ID NO: 162 - RNA, 21 nt, synthetic construct
  source 1..21: mol_type = other RNA
aaaaaggtgggagactggggg

SEQ ID NO: 163 - RNA, 21 nt, synthetic construct
  source 1..21: mol_type = other RNA
agaaaaggtgggagactgggg

SEQ ID NO: 164 - RNA, 21 nt, synthetic construct
  source 1..21: mol_type = other RNA
aagaaaaggtgggagactggg

SEQ ID NO: 165 - RNA, 21 nt, synthetic construct
  source 1..21: mol_type = other RNA
aaagaaaaggtgggagactgg

SEQ ID NO: 166 - RNA, 21 nt, synthetic construct
  source 1..21: mol_type = other RNA
agaagaaaaggtgggagactg

SEQ ID NO: 167 - RNA, 21 nt, synthetic construct
  source 1..21: mol_type = other RNA
tagaagaaaaggtgggagact

SEQ ID NO: 168 - RNA, 21 nt, synthetic construct
  source 1..21: mol_type = other RNA
tattagaagaaaaggtgggag

SEQ ID NO: 169 - RNA, 21 nt, synthetic construct
  source 1..21: mol_type = other RNA
tcattagaagaaaaggtggga

SEQ ID NO: 170 - RNA, 21 nt, synthetic construct
  source 1..21: mol_type = other RNA
actcattagaagaaaaggtgg

SEQ ID NO: 171 - RNA, 21 nt, synthetic construct
  source 1..21: mol_type = other RNA
aactcattagaagaaaaggtg

SEQ ID NO: 172 - RNA, 21 nt, synthetic construct
  source 1..21: mol_type = other RNA
tgactcattagaagaaaaggt

SEQ ID NO: 173 - RNA, 21 nt, synthetic construct
  source 1..21: mol_type = other RNA
tcgactcattagaagaaaagg

SEQ ID NO: 174 - RNA, 21 nt, synthetic construct
  source 1..21: mol_type = other RNA
atcgactcattagaagaaaag

SEQ ID NO: 175 - RNA, 21 nt, synthetic construct
  source 1..21: mol_type = other RNA
agtcgactcattagaagaaaa

SEQ ID NO: 176 - RNA, 23 nt, synthetic construct
  source 1..23: mol_type = other RNA
aaggtgggagactgggggtgaca

SEQ ID NO: 177 - RNA, 23 nt, synthetic construct
  source 1..23: mol_type = other RNA
aaaggtgggagactgggggtgac

SEQ ID NO: 178 - RNA, 23 nt, synthetic construct
  source 1..23: mol_type = other RNA
aaaaggtgggagactgggggtga

SEQ ID NO: 179 - RNA, 23 nt, synthetic construct
  source 1..23: mol_type = other RNA
aaaaaggtgggagactgggggtg

SEQ ID NO: 180 - RNA, 23 nt, synthetic construct
  source 1..23: mol_type = other RNA
agaaaaggtgggagactgggggt

SEQ ID NO: 181 - RNA, 23 nt, synthetic construct
  source 1..23: mol_type = other RNA
aagaaaaggtgggagactggggg

SEQ ID NO: 182 - RNA, 23 nt, synthetic construct
  source 1..23: mol_type = other RNA
aaagaaaaggtgggagactgggg

SEQ ID NO: 183 - RNA, 23 nt, synthetic construct
  source 1..23: mol_type = other RNA
agaagaaaaggtgggagactggg

SEQ ID NO: 184 - RNA, 23 nt, synthetic construct
  source 1..23: mol_type = other RNA
tagaagaaaaggtgggagactgg

SEQ ID NO: 185 - RNA, 23 nt, synthetic construct
  source 1..23: mol_type = other RNA
tattagaagaaaaggtgggagac

SEQ ID NO: 186 - RNA, 23 nt, synthetic construct
  source 1..23: mol_type = other RNA
tcattagaagaaaaggtgggaga

SEQ ID NO: 187 - RNA, 23 nt, synthetic construct
  source 1..23: mol_type = other RNA
actcattagaagaaaaggtggga

SEQ ID NO: 188 - RNA, 23 nt, synthetic construct
  source 1..23: mol_type = other RNA
aactcattagaagaaaaggtggg

SEQ ID NO: 189 - RNA, 23 nt, synthetic construct
  source 1..23: mol_type = other RNA
tgactcattagaagaaaaggtgg

SEQ ID NO: 190 - RNA, 23 nt, synthetic construct
  source 1..23: mol_type = other RNA
tcgactcattagaagaaaaggtg

SEQ ID NO: 191 - RNA, 23 nt, synthetic construct
  source 1..23: mol_type = other RNA
atcgactcattagaagaaaaggt

SEQ ID NO: 192 - RNA, 23 nt, synthetic construct
  source 1..23: mol_type = other RNA
agtcgactcattagaagaaaagg

SEQ ID NO: 193 - RNA, 22 nt, synthetic construct
  source 1..22: mol_type = other RNA
tacttagaccaaggagaaactt

SEQ ID NO: 194 - RNA, 22 nt, synthetic construct
  source 1..22: mol_type = other RNA
aagcgtgggaggaccacaggtt

SEQ ID NO: 195 - RNA, 22 nt, synthetic construct
  source 1..22: mol_type = other RNA
aaggtggaaggggtgtatgttt

SEQ ID NO: 196 - RNA, 22 nt, synthetic construct
  source 1..22: mol_type = other RNA
agaaggggtgtatgtacacctt

SEQ ID NO: 197 - RNA, 22 nt, synthetic construct
  source 1..22: mol_type = other RNA
tggaaagtgagaccctccactt

SEQ ID NO: 198 - RNA, 22 nt, synthetic construct
  source 1..22: mol_type = other RNA
ttcccttggaagtggacgtatt

SEQ ID NO: 199 - RNA, 22 nt, synthetic construct
  source 1..22: mol_type = other RNA
aaagaaaaggtgggagactgtt

SEQ ID NO: 200 - RNA, 22 nt, synthetic construct
  source 1..22: mol_type = other RNA
aagagcgtgggaggaccacatt

SEQ ID NO: 201 - RNA, 23 nt, synthetic construct
  source 1..23: mol_type = other RNA
  misc_feature 12: note = T
aaaaatgctgttcagcacctccc

SEQ ID NO: 202 - RNA, 23 nt, synthetic construct
  source 1..23: mol_type = other RNA
  misc_feature 1: note = I, as defined in the specification
nttgctggaaagtgagaccctcc

SEQ ID NO: 203 - RNA, 23 nt, synthetic construct
  source 1..23: mol_type = other RNA
  misc_feature 6: note = T
  misc_feature 1: note = I, as defined in the specification
nttgctggaaagtgagaccctcc

SEQ ID NO: 204 - RNA, 23 nt, synthetic construct
  source 1..23: mol_type = other RNA
  misc_feature 2: note = T
  misc_feature 1: note = I, as defined in the specification
nttgctggaaagtgagaccctcc

SEQ ID NO: 205 - RNA, 23 nt, synthetic construct
  source 1..23: mol_type = other RNA
  misc_feature 1: note = I, as defined in the specification
naaaatgctgttcagcacctccc

SEQ ID NO: 206 - RNA, 23 nt, synthetic construct
  source 1..23: mol_type = other RNA
  misc_feature 6: note = T
  misc_feature 1: note = I, as defined in the specification
naaaatgctgttcagcacctccc

SEQ ID NO: 207 - RNA, 22 nt, synthetic construct
  source 1..22: mol_type = other RNA
  misc_feature 22: note = I, as defined in the specification
ttcattagaagaaaaggtggtn

SEQ ID NO: 208 - RNA, 20 nt, synthetic construct
  source 1..20: mol_type = other RNA
gcaccttttcttctaatgaa

SEQ ID NO: 209 - RNA, 22 nt, synthetic construct
  source 1..22: mol_type = other RNA
  misc_feature 22: note = I, as defined in the specification
ttcattagaagaaaaggtgctn

SEQ ID NO: 210 - RNA, 22 nt, synthetic construct
  source 1..22: mol_type = other RNA
  misc_feature 17: note = I, as defined in the specification
ttcattagaagaaaagntggtt

SEQ ID NO: 211 - RNA, 22 nt, synthetic construct
  source 1..22: mol_type = other RNA
  misc_feature 20: note = I, as defined in the specification
ttcattagaagaaaaggtgntt

SEQ ID NO: 212 - RNA, 22 nt, synthetic construct
  source 1..22: mol_type = other RNA
  misc_feature 21: note = T
aaaaatgctgttcagcaccttt

SEQ ID NO: 213 - RNA, 22 nt, synthetic construct
  source 1..22: mol_type = other RNA
  misc_feature 12: note = T
aaaaatgctgttcagcaccttt

SEQ ID NO: 214 - RNA, 22 nt, synthetic construct
  source 1..22: mol_type = other RNA
  misc_feature 21: note = T
taaaatgctgttcagcaccttt

SEQ ID NO: 215 - RNA, 22 nt, synthetic construct
  source 1..22: mol_type = other RNA
  misc_feature 12: note = T
taaaatgctgttcagcaccttt

SEQ ID NO: 216 - RNA, 21 nt, synthetic construct
  source 1..21: mol_type = other RNA
  misc_feature 20: note = T
aaaaatgctgttcagcacctt

SEQ ID NO: 217 - RNA, 21 nt, synthetic construct
  source 1..21: mol_type = other RNA
  misc_feature 12: note = T
aaaaatgctgttcagcacctt

SEQ ID NO: 218 - RNA, 21 nt, synthetic construct
  source 1..21: mol_type = other RNA
  misc_feature 20: note = T
taaaatgctgttcagcacctt

SEQ ID NO: 219 - RNA, 21 nt, synthetic construct
  source 1..21: mol_type = other RNA
  misc_feature 12: note = T
taaaatgctgttcagcacctt

SEQ ID NO: 220 - RNA, 22 nt, synthetic construct
  source 1..22: mol_type = other RNA
  misc_feature 21: note = T
attgctggaaagtgagaccctt

SEQ ID NO: 221 - RNA, 20 nt, synthetic construct
  source 1..20: mol_type = other RNA
  misc_feature 6: note = T
gggtctcactttccagcaat

SEQ ID NO: 222 - RNA, 22 nt, synthetic construct
  source 1..22: mol_type = other RNA
  misc_feature 2: note = T
attgctggaaagtgagaccctt

SEQ ID NO: 223 - RNA, 22 nt, synthetic construct
  source 1..22: mol_type = other RNA
  misc_feature 21: note = T
taagctgttgggtagactcttt

SEQ ID NO: 224 - RNA, 20 nt, synthetic construct
  source 1..20: mol_type = other RNA
  misc_feature 1: note = T
tctcccaccttttcttctaa

SEQ ID NO: 225 - RNA, 22 nt, synthetic construct
  source 1..22: mol_type = other RNA
  misc_feature 21: note = T
ttagaagaaaaggtgggagatt

SEQ ID NO: 226 - RNA, 22 nt, synthetic construct
  source 1..22: mol_type = other RNA
  misc_feature 2: note = T
ttagaagaaaaggtgggagatt

SEQ ID NO: 227 - RNA, 22 nt, synthetic construct
  source 1..22: mol_type = other RNA
  misc_feature 21: note = T
tttagaagaaaaggtgggagtt

SEQ ID NO: 228 - RNA, 22 nt, synthetic construct
  source 1..22: mol_type = other RNA
  misc_feature 2: note = T
tttagaagaaaaggtgggagtt

SEQ ID NO: 229 - RNA, 22 nt, synthetic construct
  source 1..22: mol_type = other RNA
  misc_feature 21: note = T
ttcattagaagaaaaggtggtt

SEQ ID NO: 230 - RNA, 22 nt, synthetic construct
  source 1..22: mol_type = other RNA
  misc_feature 2: note = T
  misc_feature 5: note = T
ttcattagaagaaaaggtggtt

SEQ ID NO: 231 - RNA, 21 nt, synthetic construct
  source 1..21: mol_type = other RNA
  misc_feature 20: note = T
ttcattagaagaaaaggtgtt

SEQ ID NO: 232 - RNA, 21 nt, synthetic construct
  source 1..21: mol_type = other RNA
  misc_feature 2: note = T
ttcattagaagaaaaggtgtt

SEQ ID NO: 233 - RNA, 23 nt, synthetic construct
  source 1..23: mol_type = other RNA
  misc_feature 22: note = T
taagctgttgggtagactctgtg

SEQ ID NO: 234 - RNA, 20 nt, synthetic construct
  source 1..20: mol_type = other RNA
  misc_feature 6: note = T
ccaccttttcttctaatgaa

SEQ ID NO: 235 - RNA, 23 nt, synthetic construct
  source 1..23: mol_type = other RNA
  misc_feature 6: note = T
attgctggaaagtgagaccctcc

SEQ ID NO: 236 - RNA, 22 nt, synthetic construct
  source 1..22: mol_type = other RNA
  misc_feature 6: note = T
ttcattagaagaaaaggtggtt

SEQ ID NO: 237 - RNA, 21 nt, synthetic construct
  source 1..21: mol_type = other RNA
  misc_feature 6: note = T
ttcattagaagaaaaggtgtt

SEQ ID NO: 238 - RNA, 22 nt, synthetic construct
  source 1..22: mol_type = other RNA
  misc_feature 5: note = T
ttcattagaagaaaaggtggtt

SEQ ID NO: 239 - RNA, 22 nt, synthetic construct
  source 1..22: mol_type = other RNA
  misc_feature 5: note = I, as defined in the specification
ttagnagaaaaggtgggagatt

SEQ ID NO: 240 - RNA, 22 nt, synthetic construct
  source 1..22: mol_type = other RNA
  misc_feature 5: note = I, as defined in the specification
tttanaagaaaaggtgggagtt

SEQ ID NO: 241 - RNA, 22 nt, synthetic construct
  source 1..22: mol_type = other RNA
  misc_feature 5: note = I, as defined in the specification
ttcantagaagaaaaggtggtt

SEQ ID NO: 242 - RNA, 22 nt, synthetic construct
  source 1..22: mol_type = other RNA
  misc_feature 6: note = I, as defined in the specification
ttagangaaaaggtgggagatt

SEQ ID NO: 243 - RNA, 22 nt, synthetic construct
  source 1..22: mol_type = other RNA
  misc_feature 6: note = I, as defined in the specification
tttagnagaaaaggtgggagtt

SEQ ID NO: 244 - RNA, 22 nt, synthetic construct
  source 1..22: mol_type = other RNA
  misc_feature 6: note = I, as defined in the specification
ttcatnagaagaaaaggtggtt

SEQ ID NO: 245 - RNA, 22 nt, synthetic construct
  source 1..22: mol_type = other RNA
  misc_feature 7: note = I, as defined in the specification
ttagaanaaaaggtgggagatt

SEQ ID NO: 246 - RNA, 22 nt, synthetic construct
  source 1..22: mol_type = other RNA
  misc_feature 7: note = I, as defined in the specification
tttagangaaaaggtgggagtt

SEQ ID NO: 247 - RNA, 22 nt, synthetic construct
  source 1..22: mol_type = other RNA
  misc_feature 7: note = I, as defined in the specification
ttcattngaagaaaaggtggtt

SEQ ID NO: 248 - RNA, 22 nt, synthetic construct
  source 1..22: mol_type = other RNA
  misc_feature 8: note = I, as defined in the specification
ttagaagnaaaggtgggagatt

SEQ ID NO: 249 - RNA, 22 nt, synthetic construct
  source 1..22: mol_type = other RNA
  misc_feature 8: note = I, as defined in the specification
tttagaanaaaaggtgggagtt

SEQ ID NO: 250 - RNA, 22 nt, synthetic construct
  source 1..22: mol_type = other RNA
  misc_feature 8: note = I, as defined in the specification
ttcattanaagaaaaggtggtt

SEQ ID NO: 251 - RNA, 21 nt, synthetic construct
  source 1..21: mol_type = other RNA
gtcatccacaatgagagtaca

SEQ ID NO: 252 - RNA, 23 nt, synthetic construct
  source 1..23: mol_type = other RNA
  misc_feature 5: note = I, as defined in the specification
tgtantctcattgtggatgacga

SEQ ID NO: 253 - RNA, 23 nt, synthetic construct
  source 1..23: mol_type = other RNA
  misc_feature 6: note = I, as defined in the specification
tgtacnctcattgtggatgacga

SEQ ID NO: 254 - RNA, 23 nt, synthetic construct
  source 1..23: mol_type = other RNA
  misc_feature 7: note = I, as defined in the specification
tgtactntcattgtggatgacga

SEQ ID NO: 255 - RNA, 23 nt, synthetic construct
  source 1..23: mol_type = other RNA
  misc_feature 8: note = I, as defined in the specification
tgtactcncattgtggatgacga

SEQ ID NO: 256 - RNA, 22 nt, synthetic construct
  source 1..22: mol_type = other RNA
  misc_feature 5: note = B, as defined in the specification
ttagnagaaaaggtgggagatt

SEQ ID NO: 257 - RNA, 22 nt, synthetic construct
  source 1..22: mol_type = other RNA
  misc_feature 5: note = B, as defined in the specification
tttanaagaaaaggtgggagtt

SEQ ID NO: 258 - RNA, 22 nt, synthetic construct
  source 1..22: mol_type = other RNA
  misc_feature 5: note = B, as defined in the specification
ttcantagaagaaaaggtggtt

SEQ ID NO: 259 - RNA, 22 nt, synthetic construct
  source 1..22: mol_type = other RNA
  misc_feature 6: note = B, as defined in the specification
ttagangaaaaggtgggagatt

SEQ ID NO: 260 - RNA, 22 nt, synthetic construct
  source 1..22: mol_type = other RNA
  misc_feature 6: note = B, as defined in the specification
tttagnagaaaaggtgggagtt

SEQ ID NO: 261 - RNA, 22 nt, synthetic construct
  source 1..22: mol_type = other RNA
  misc_feature 6: note = B, as defined in the specification
ttcatnagaagaaaaggtggtt

SEQ ID NO: 262 - RNA, 22 nt, synthetic construct
  source 1..22: mol_type = other RNA
  misc_structure 7: note = B, as defined in the specification
ttagaanaaaaggtgggagatt

SEQ ID NO: 263 - RNA, 22 nt, synthetic construct
  source 1..22: mol_type = other RNA
  misc_feature 7: note = B, as defined in the specification
tttagangaaaaggtgggagtt

SEQ ID NO: 264 - RNA, 22 nt, synthetic construct
  source 1..22: mol_type = other RNA
  misc_feature 7: note = B, as defined in the specification
ttcattngaagaaaaggtggtt

SEQ ID NO: 265 - RNA, 22 nt, synthetic construct
  source 1..22: mol_type = other RNA
  misc_feature 8: note = B, as defined in the specification
ttagaagnaaaggtgggagatt

SEQ ID NO: 266 - RNA, 22 nt, synthetic construct
  source 1..22: mol_type = other RNA
  misc_feature 8: note = B, as defined in the specification
tttagaanaaaaggtgggagtt

SEQ ID NO: 267 - RNA, 22 nt, synthetic construct
  source 1..22: mol_type = other RNA
  misc_feature 8: note = B, as defined in the specification
ttcattanaagaaaaggtggtt

SEQ ID NO: 268 - RNA, 22 nt, synthetic construct
  source 1..22: mol_type = other RNA
  misc_feature 5: note = X, as defined in the specification
ttagnagaaaaggtgggagatt

SEQ ID NO: 269 - RNA, 22 nt, synthetic construct
  source 1..22: mol_type = other RNA
  misc_feature 5: note = X, as defined in the specification
tttanaagaaaaggtgggagtt

SEQ ID NO: 270 - RNA, 22 nt, synthetic construct
  source 1..22: mol_type = other RNA
  misc_feature 5: note = X, as defined in the specification
ttcantagaagaaaaggtggtt

SEQ ID NO: 271 - RNA, 22 nt, synthetic construct
  source 1..22: mol_type = other RNA
  misc_feature 6: note = X, as defined in the specification
ttagangaaaaggtgggagatt

SEQ ID NO: 272 - RNA, 22 nt, synthetic construct
  source 1..22: mol_type = other RNA
  misc_feature 6: note = X, as defined in the specification
tttagnagaaaaggtgggagtt

SEQ ID NO: 273 - RNA, 22 nt, synthetic construct
  source 1..22: mol_type = other RNA
  misc_feature 6: note = X, as defined in the specification
ttcatnagaagaaaaggtggtt

SEQ ID NO: 274 - RNA, 22 nt, synthetic construct
  source 1..22: mol_type = other RNA
  misc_feature 7: note = X, as defined in the specification
ttagaanaaaaggtgggagatt

SEQ ID NO: 275 - RNA, 22 nt, synthetic construct
  source 1..22: mol_type = other RNA
  misc_feature 7: note = X, as defined in the specification
tttagangaaaaggtgggagtt

SEQ ID NO: 276 - RNA, 22 nt, synthetic construct
  source 1..22: mol_type = other RNA
  misc_feature 7: note = X, as defined in the specification
ttcattngaagaaaaggtggtt

SEQ ID NO: 277 - RNA, 22 nt, synthetic construct
  source 1..22: mol_type = other RNA
  misc_feature 8: note = X, as defined in the specification
ttagaagnaaaggtgggagatt

SEQ ID NO: 278 - RNA, 22 nt, synthetic construct
  source 1..22: mol_type = other RNA
  misc_feature 8: note = X, as defined in the specification
tttagaanaaaaggtgggagtt

SEQ ID NO: 279 - RNA, 22 nt, synthetic construct
  source 1..22: mol_type = other RNA
  misc_feature 8: note = X, as defined in the specification
ttcattanaagaaaaggtggtt

SEQ ID NO: 280 - RNA, 22 nt, synthetic construct
  source 1..22: mol_type = other RNA
tttaaaagaaaaggtgggagtt

SEQ ID NO: 281 - RNA, 22 nt, synthetic construct
  source 1..22: mol_type = other RNA
ttcaatagaagaaaaggtggtt

SEQ ID NO: 282 - RNA, 22 nt, synthetic construct
  source 1..22: mol_type = other RNA
ttcataagaagaaaaggtggtt

SEQ ID NO: 283 - RNA, 22 nt, synthetic construct
  source 1..22: mol_type = other RNA
ttagaaaaaaaggtgggagatt

SEQ ID NO: 284 - RNA, 22 nt, synthetic construct
  source 1..22: mol_type = other RNA
tttagaaaaaaaggtgggagtt

SEQ ID NO: 285 - RNA, 22 nt, synthetic construct
  source 1..22: mol_type = other RNA
ttcattaaaagaaaaggtggtt

SEQ ID NO: 286 - RNA, 23 nt, synthetic construct
  source 1..23: mol_type = other RNA
  misc_feature 2: note = T
ttgtgggctctctctcatccggg

SEQ ID NO: 287 - RNA, 22 nt, synthetic construct
  source 1..22: mol_type = other RNA
  misc_feature 22: note = I, as defined in the specification
ttagaagaaaaggtgggagatn

SEQ ID NO: 288 - RNA, 22 nt, synthetic construct
  source 1..22: mol_type = other RNA
  misc_feature 22: note = I, as defined in the specification
tttagaagaaaaggtgggagtn

SEQ ID NO: 289 - RNA, 22 nt, synthetic construct
  source 1..22: mol_type = other RNA
  misc_feature 21: note = I, as defined in the specification
ttagaagaaaaggtgggagant

SEQ ID NO: 290 - RNA, 22 nt, synthetic construct
  source 1..22: mol_type = other RNA
  misc_feature 21: note = I, as defined in the specification
tttagaagaaaaggtgggagnt

SEQ ID NO: 291 - RNA, 22 nt, synthetic construct
  source 1..22: mol_type = other RNA
  misc_feature 21: note = I, as defined in the specification
ttcattagaagaaaaggtggnt

SEQ ID NO: 292 - RNA, 19 nt, synthetic construct
  source 1..19: mol_type = other RNA
  misc_feature 1: note = T
tcccaccttttcttctaaa

SEQ ID NO: 293 - RNA, 21 nt, synthetic construct
  source 1..21: mol_type = other RNA
  misc_feature 21: note = I, as defined in the specification
ttagaagaaaaggtgggagtn

SEQ ID NO: 294 - RNA, 21 nt, synthetic construct
  source 1..21: mol_type = other RNA
  misc_feature 21: note = I, as defined in the specification
tttagaagaaaaggtgggatn

SEQ ID NO: 295 - RNA, 21 nt, synthetic construct
  source 1..21: mol_type = other RNA
  misc_feature 21: note = I, as defined in the specification
ttcattagaagaaaaggtgtn

SEQ ID NO: 296 - RNA, 21 nt, synthetic construct
  source 1..21: mol_type = other RNA
  misc_feature 20: note = I, as defined in the specification
ttagaagaaaaggtgggagnt

SEQ ID NO: 297 - RNA, 21 nt, synthetic construct
  source 1..21: mol_type = other RNA
  misc_feature 20: note = I, as defined in the specification
tttagaagaaaaggtgggant

SEQ ID NO: 298 - RNA, 21 nt, synthetic construct
  source 1..21: mol_type = other RNA
  misc_feature 20: note = I, as defined in the specification
ttcattagaagaaaaggtgnt

SEQ ID NO: 299 - RNA, 22 nt, synthetic construct
  source 1..22: mol_type = other RNA
ttcattagaagaaaaggtggga

SEQ ID NO: 300 - RNA, 21 nt, synthetic construct
  source 1..21: mol_type = other RNA
ttcattagaagaaaaggtggg

SEQ ID NO: 301 - RNA, 22 nt, synthetic construct
  source 1..22: mol_type = other RNA
  misc_feature 1: note = B, as defined in the specification
ntcattagaagaaaaggtggga

SEQ ID NO: 302 - RNA, 21 nt, synthetic construct
  source 1..21: mol_type = other RNA
  misc_feature 1: note = B, as defined in the specification
ntcattagaagaaaaggtggg

SEQ ID NO: 303 - RNA, 22 nt, synthetic construct
  source 1..22: mol_type = other RNA
  misc_feature 1: note = B, as defined in the specification
ntcattagaagaaaaggtggtt

SEQ ID NO: 304 - RNA, 21 nt, synthetic construct
  source 1..21: mol_type = other RNA
  misc_feature 1: note = B, as defined in the specification
ntcattagaagaaaaggtgtt

SEQ ID NO: 305 - RNA, 22 nt, synthetic construct
  source 1..22: mol_type = other RNA
  misc_feature 21: note = I, as defined in the specification
  misc_feature 1: note = B, as defined in the specification
ntcattagaagaaaaggtggnt

SEQ ID NO: 306 - RNA, 21 nt, synthetic construct
  source 1..21: mol_type = other RNA
  misc_feature 20: note = I, as defined in the specification
  misc_feature 1: note = B, as defined in the specification
ntcattagaagaaaaggtgnt

SEQ ID NO: 307 - RNA, 22 nt, synthetic construct
  source 1..22: mol_type = other RNA
  misc_feature 22: note = I, as defined in the specification
  misc_feature 1: note = B, as defined in the specification
ntcattagaagaaaaggtggtn

SEQ ID NO: 308 - RNA, 21 nt, synthetic construct
  source 1..21: mol_type = other RNA
  misc_feature 21: note = I, as defined in the specification
  misc_feature 1: note = B, as defined in the specification
ntcattagaagaaaaggtgtn

SEQ ID NO: 309 - RNA, 22 nt, synthetic construct
  source 1..22: mol_type = other RNA
  misc_feature 1: note = X, as defined in the specification
ntcattagaagaaaaggtggga

SEQ ID NO: 310 - RNA, 21 nt, synthetic construct
  source 1..21: mol_type = other RNA
  misc_feature 1: note = X, as defined in the specification
ntcattagaagaaaaggtggg

SEQ ID NO: 311 - RNA, 22 nt, synthetic construct
  source 1..22: mol_type = other RNA
  misc_feature 1: note = X, as defined in the specification
ntcattagaagaaaaggtggtt

SEQ ID NO: 312 - RNA, 21 nt, synthetic construct
  source 1..21: mol_type = other RNA
  misc_feature 1: note = X, as defined in the specification
ntcattagaagaaaaggtgtt

SEQ ID NO: 313 - RNA, 22 nt, synthetic construct
  source 1..22: mol_type = other RNA
  misc_feature 21: note = I, as defined in the specification
  misc_feature 1: note = X, as defined in the specification
ntcattagaagaaaaggtggnt

SEQ ID NO: 314 - RNA, 21 nt, synthetic construct
  source 1..21: mol_type = other RNA
  misc_feature 20: note = I, as defined in the specification
  misc_feature 1: note = X, as defined in the specification
ntcattagaagaaaaggtgnt

SEQ ID NO: 315 - RNA, 22 nt, synthetic construct
  source 1..22: mol_type = other RNA
  misc_feature 22: note = I, as defined in the specification
  misc_feature 1: note = X, as defined in the specification
ntcattagaagaaaaggtggtn

SEQ ID NO: 316 - RNA, 21 nt, synthetic construct
  source 1..21: mol_type = other RNA
  misc_feature 21: note = I, as defined in the specification
  misc_feature 1: note = X, as defined in the specification
ntcattagaagaaaaggtgtn

SEQ ID NO: 317 - RNA, 22 nt, synthetic construct
  source 1..22: mol_type = other RNA
  misc_feature 2: note = T
  misc_feature 5: note = T
ttcattagaagaaaaggtggga

SEQ ID NO: 318 - RNA, 21 nt, synthetic construct
  source 1..21: mol_type = other RNA
  misc_feature 2: note = T
  misc_feature 5: note = T
ttcattagaagaaaaggtggg

SEQ ID NO: 319 - RNA, 21 nt, synthetic construct
  source 1..21: mol_type = other RNA
  misc_feature 2: note = T
  misc_feature 5: note = T
ttcattagaagaaaaggtgtt

SEQ ID NO: 320 - RNA, 22 nt, synthetic construct
  source 1..22: mol_type = other RNA
  misc_feature 2: note = T
  misc_feature 5: note = T
  misc_feature 1: note = B, as defined in the specification
ntcattagaagaaaaggtggga

SEQ ID NO: 321 - RNA, 21 nt, synthetic construct
  source 1..21: mol_type = other RNA
  misc_feature 2: note = T
  misc_feature 5: note = T
  misc_feature 1: note = B, as defined in the specification
ntcattagaagaaaaggtggg

SEQ ID NO: 322 - RNA, 22 nt, synthetic construct
  source 1..22: mol_type = other RNA
  misc_feature 2: note = T
  misc_feature 5: note = T
  misc_feature 1: note = B, as defined in the specification
ntcattagaagaaaaggtggtt

SEQ ID NO: 323 - RNA, 21 nt, synthetic construct
  source 1..21: mol_type = other RNA
  misc_feature 2: note = T
  misc_feature 5: note = T
  misc_feature 1: note = B, as defined in the specification
ntcattagaagaaaaggtgtt

SEQ ID NO: 324 - RNA, 22 nt, synthetic construct
  source 1..22: mol_type = other RNA
  misc_feature 2: note = T
  misc_feature 5: note = T
  misc_feature 1: note = X, as defined in the specification
ntcattagaagaaaaggtggga

SEQ ID NO: 325 - RNA, 21 nt, synthetic construct
  source 1..21: mol_type = other RNA
  misc_feature 2: note = T
  misc_feature 5: note = T
  misc_feature 1: note = X, as defined in the specification
ntcattagaagaaaaggtggg

SEQ ID NO: 326 - RNA, 22 nt, synthetic construct
  source 1..22: mol_type = other RNA
  misc_feature 2: note = T
  misc_feature 5: note = T
  misc_feature 1: note = X, as defined in the specification
ntcattagaagaaaaggtggtt

SEQ ID NO: 327 - RNA, 21 nt, synthetic construct
  source 1..21: mol_type = other RNA
  misc_feature 2: note = T
  misc_feature 5: note = T
  misc_feature 1: note = X, as defined in the specification
ntcattagaagaaaaggtgtt

SEQ ID NO: 328 - RNA, 22 nt, synthetic construct
  source 1..22: mol_type = other RNA
  misc_feature 2: note = T
  misc_feature 5: note = T
  misc_feature 21: note = I, as defined in the specification
ttcattagaagaaaaggtggnt

SEQ ID NO: 329 - RNA, 21 nt, synthetic construct
  source 1..21: mol_type = other RNA
  misc_feature 2: note = T
  misc_feature 5: note = T
  misc_feature 20: note = I, as defined in the specification
ttcattagaagaaaaggtgnt

SEQ ID NO: 330 - RNA, 22 nt, synthetic construct
  source 1..22: mol_type = other RNA
  misc_feature 2: note = T
  misc_feature 5: note = T
  misc_feature 21: note = I, as defined in the specification
  misc_feature 1: note = B, as defined in the specification
ntcattagaagaaaaggtggnt

SEQ ID NO: 331 - RNA, 21 nt, synthetic construct
  source 1..21: mol_type = other RNA
  misc_feature 2: note = T
  misc_feature 5: note = T
  misc_feature 20: note = I, as defined in the specification
  misc_feature 1: note = B, as defined in the specification
ntcattagaagaaaaggtgnt

SEQ ID NO: 332 - RNA, 22 nt, synthetic construct
  source 1..22: mol_type = other RNA
  misc_feature 2: note = T
  misc_feature 5: note = T
  misc_feature 21: note = I, as defined in the specification
  misc_feature 1: note = X, as defined in the specification
ntcattagaagaaaaggtggnt

SEQ ID NO: 333 - RNA, 21 nt, synthetic construct
  source 1..21: mol_type = other RNA
  misc_feature 2: note = T
  misc_feature 5: note = T
  misc_feature 20: note = I, as defined in the specification
  misc_feature 1: note = X, as defined in the specification
ntcattagaagaaaaggtgnt

SEQ ID NO: 334 - RNA, 22 nt, synthetic construct
  source 1..22: mol_type = other RNA
  misc_feature 22: note = I, as defined in the specification
  misc_feature 2: note = T
  misc_feature 5: note = T
ttcattagaagaaaaggtggtn

SEQ ID NO: 335 - RNA, 21 nt, synthetic construct
  source 1..21: mol_type = other RNA
  misc_feature 21: note = I, as defined in the specification
  misc_feature 2: note = T
  misc_feature 5: note = T
ttcattagaagaaaaggtgtn

SEQ ID NO: 336 - RNA, 22 nt, synthetic construct
  source 1..22: mol_type = other RNA
  misc_feature 22: note = I, as defined in the specification
  misc_feature 1: note = B, as defined in the specification
  misc_feature 2: note = T
  misc_feature 5: note = T
ntcattagaagaaaaggtggtn

SEQ ID NO: 337 - RNA, 21 nt, synthetic construct
  source 1..21: mol_type = other RNA
  misc_feature 21: note = I, as defined in the specification
  misc_feature 1: note = B, as defined in the specification
  misc_feature 2: note = T
  misc_feature 5: note = T
ntcattagaagaaaaggtgtn

SEQ ID NO: 338 - RNA, 22 nt, synthetic construct
  source 1..22: mol_type = other RNA
  misc_feature 22: note = I, as defined in the specification
  misc_feature 1: note = X, as defined in the specification
  misc_feature 2: note = T
  misc_feature 5: note = T
ntcattagaagaaaaggtggtn

SEQ ID NO: 339 - RNA, 21 nt, synthetic construct
  source 1..21: mol_type = other RNA
  misc_feature 21: note = I, as defined in the specification
  misc_feature 1: note = X, as defined in the specification
  misc_feature 2: note = T
  misc_feature 5: note = T
ntcattagaagaaaaggtgtn

SEQ ID NO: 340 - RNA, 20 nt, synthetic construct
  source 1..20: mol_type = other RNA
ttcattagaagaaaaggtgg

SEQ ID NO: 341 - RNA, 19 nt, synthetic construct
  source 1..19: mol_type = other RNA
ttcattagaagaaaaggtg

SEQ ID NO: 342 - RNA, 21 nt, synthetic construct
  source 1..21: mol_type = other RNA
cccaccttttcttctaatgaa

SEQ ID NO: 343 - RNA, 23 nt, synthetic construct
  source 1..23: mol_type = other RNA
ttcattagaagaaaaggtgggtt

SEQ ID NO: 344 - RNA, 23 nt, synthetic construct
  source 1..23: mol_type = other RNA
  misc_feature 22: note = T
  misc_feature 23: note = T
ttcattagaagaaaaggtgggtt

SEQ ID NO: 345 - RNA, 22 nt, synthetic construct
  source 1..22: mol_type = other RNA
  misc_feature 21: note = T
  misc_feature 22: note = T
ttcattagaagaaaaggtggtt

SEQ ID NO: 346 - RNA, 21 nt, synthetic construct
  source 1..21: mol_type = other RNA
  misc_feature 20: note = T
  misc_feature 21: note = T
ttcattagaagaaaaggtgtt

SEQ ID NO: 347 - RNA, 23 nt, synthetic construct
  source 1..23: mol_type = other RNA
ttcattagaagaaaaggtgggag

SEQ ID NO: 348 - RNA, 23 nt, synthetic construct
  source 1..23: mol_type = other RNA
  misc_feature 6: note = T
tgtactctcattgtggatgacga

SEQ ID NO: 349 - RNA, 23 nt, synthetic construct
  source 1..23: mol_type = other RNA
aatttagaccaaggagaaacgtc

SEQ ID NO: 350 - RNA, 21 nt, synthetic construct
  source 1..21: mol_type = other RNA
cgtttctccttggtctaaatt

SEQ ID NO: 351 - RNA, 23 nt, synthetic construct
  source 1..23: mol_type = other RNA
cacttagaccaaggagaaacgtc